European Patent Application EP 4 442 275 A1, published October 9, 2024. Title: Antibodies. Applicant: ModiQuest B. V. Application EP. The sequence listing filed with the application follows.

SEQUENCE LISTING (120 sequences)

SEQ ID NO: 1 - protein, 116 aa, Mus musculus
DVQLQESGPGLVKPSQSLSLTCSVTGYSITSDYYWHWIRQFPGNKLEWMGYISYDGSNNYNPSLKNRISITRDTSKNQFFLKLNSVTTEDTATYYCARDDDAMDYWGQGTSVTVSS

SEQ ID NO: 2 - protein, 25 aa, Mus musculus
DVQLQESGPGLVKPSQSLSLTCSVT

SEQ ID NO: 3 - protein, 9 aa, Mus musculus
GYSITSDYY

SEQ ID NO: 4 - protein, 17 aa, Mus musculus
WHWIRQFPGNKLEWMGY

SEQ ID NO: 5 - protein, 7 aa, Mus musculus
ISYDGSN

SEQ ID NO: 6 - protein, 38 aa, Mus musculus
NYNPSLKNRISITRDTSKNQFFLKLNSVTTEDTATYYC

SEQ ID NO: 7 - protein, 9 aa, Mus musculus
ARDDDAMDY

SEQ ID NO: 8 - protein, 11 aa, Mus musculus
WGQGTSVTVSS

SEQ ID NO: 9 - protein, 107 aa, Mus musculus
DIQMTQTTSSLSASLGDRVTISCRASQDISNYLNWYQQKPDGTVKLLIYYTSRLHSGVPSRFSGSGSGTDYSLTISNLEQEDIATYFCQQGNTLPPTFGGGTKLEIK

SEQ ID NO: 10 - protein, 26 aa, Mus musculus
DIQMTQTTSSLSASLGDRVTISCRAS

SEQ ID NO: 11 - protein, 6 aa, Mus musculus
QDISNY

SEQ ID NO: 12 - protein, 17 aa, Mus musculus
LNWYQQKPDGTVKLLIY

SEQ ID NO: 13 - skipped

SEQ ID NO: 14 - protein, 36 aa, Mus musculus
RLHSGVPSRFSGSGSGTDYSLTISNLEQEDIATYFC

SEQ ID NO: 15 - protein, 9 aa, Mus musculus
QQGNTLPPT

SEQ ID NO: 16 - protein, 10 aa, Mus musculus
FGGGTKLEIK

SEQ ID NO: 17 - protein, 116 aa, synthetic construct
QVQLQESGPGLVKPSETLSLTCAVSGYSITSDYYWHWIRQPPGKGLEWMGYISYDGSNNYNPSLKSRVTISVDTSKNQFSLKLSSVTAADTAVYYCARDDDAMDYWGQGTLVTVSS

SEQ ID NO: 18 - protein, 25 aa, synthetic construct
QVQLQESGPGLVKPSETLSLTCAVS

SEQ ID NO: 19 - protein, 9 aa, synthetic construct
GYSITSDYY

SEQ ID NO: 20 - protein, 17 aa, synthetic construct
WHWIRQPPGKGLEWMGY

SEQ ID NO: 21 - protein, 7 aa, synthetic construct
ISYDGSN

SEQ ID NO: 22 - protein, 38 aa, synthetic construct
NYNPSLKSRVTISVDTSKNQFSLKLSSVTAADTAVYYC

SEQ ID NO: 23 - protein, 9 aa, synthetic construct
ARDDDAMDY

SEQ ID NO: 24 - protein, 11 aa, synthetic construct
WGQGTLVTVSS

SEQ ID NO: 25 - protein, 116 aa, synthetic construct
DVQLQESGPGLVKPSETLSLTCAVSGYSITSDYYWHWIRQPPGKGLEWMGYISYDGSNNYNPSLKSRVTISVDTSKNQFSLKLSSVTAADTAVYYCARDDDAMDYWGQGTLVTVSS

SEQ ID NO: 26 - protein, 25 aa, synthetic construct
DVQLQESGPGLVKPSETLSLTCAVS

SEQ ID NO: 27 - protein, 9 aa, synthetic construct
GYSITSDYY

SEQ ID NO: 28 - protein, 17 aa, synthetic construct
WHWIRQPPGKGLEWMGY

SEQ ID NO: 29 - protein, 7 aa, synthetic construct
ISYDGSN

SEQ ID NO: 30 - protein, 38 aa, synthetic construct; identical to SEQ ID NO: 22

SEQ ID NO: 31 - protein, 9 aa, synthetic construct
ARDDDAMDY

SEQ ID NO: 32 - protein, 11 aa, synthetic construct
WGQGTLVTVSS

SEQ ID NO: 33 - protein, 116 aa, synthetic construct
DVQLQESGPGLVKPSETLSLTCAVSGYSITSDYYWHWIRQFPGKGLEWMGYISYDGSNNYNPSLKSRVTISVDTSKNQFSLKLSSVTAADTAVYYCARDDDAMDYWGQGTLVTVSS

SEQ ID NO: 34 - protein, 25 aa, synthetic construct
DVQLQESGPGLVKPSETLSLTCAVS

SEQ ID NO: 35 - protein, 9 aa, synthetic construct
GYSITSDYY

SEQ ID NO: 36 - protein, 17 aa, synthetic construct
WHWIRQFPGKGLEWMGY

SEQ ID NO: 37 - protein, 7 aa, synthetic construct
ISYDGSN

SEQ ID NO: 38 - protein, 38 aa, synthetic construct; identical to SEQ ID NO: 22

SEQ ID NO: 39 - protein, 9 aa, synthetic construct
ARDDDAMDY

SEQ ID NO: 40 - protein, 11 aa, synthetic construct
WGQGTLVTVSS

SEQ ID NO: 41 - protein, 116 aa, synthetic construct
DVQLQESGPGLVKPSETLSLTCAVSGYSITSDYYWHWIRQFPGKGLEWMGYISYDGSNNYNPSLKSRVTISRDTSKNQFSLKLSSVTAADTAVYYCARDDDAMDYWGQGTLVTVSS

SEQ ID NO: 42 - protein, 25 aa, synthetic construct
DVQLQESGPGLVKPSETLSLTCAVS

SEQ ID NO: 43 - protein, 9 aa, synthetic construct
GYSITSDYY

SEQ ID NO: 44 - protein, 17 aa, synthetic construct
WHWIRQFPGKGLEWMGY

SEQ ID NO: 45 - protein, 7 aa, synthetic construct
ISYDGSN

SEQ ID NO: 46 - protein, 38 aa, synthetic construct
NYNPSLKSRVTISRDTSKNQFSLKLSSVTAADTAVYYC

SEQ ID NO: 47 - protein, 9 aa, synthetic construct
ARDDDAMDY

SEQ ID NO: 48 - protein, 11 aa, synthetic construct
WGQGTLVTVSS

SEQ ID NO: 49 - protein, 107 aa, synthetic construct
DIQMTQSPSSLSASVGDRVTITCRASQDISNYLNWYQQKPGKAPKLLIYYTSRLHSGVPSRFSGSGSGTDFTFTISSLQPEDIATYYCQQGNTLPPTFGQGTKVEIK

SEQ ID NO: 50 - protein, 26 aa, synthetic construct [sequence omitted]

SEQ ID NO: 51 - protein, 6 aa, synthetic construct
QDISNY

SEQ ID NO: 52 - protein, 17 aa, synthetic construct
LNWYQQKPGKAPKLLIY

SEQ ID NO: 53 - skipped

SEQ ID NO: 54 - protein, 36 aa, synthetic construct [sequence omitted]

SEQ ID NO: 55 - protein, 9 aa, synthetic construct
QQGNTLPPT

SEQ ID NO: 56 - protein, 10 aa, synthetic construct
FGQGTKVEIK

SEQ ID NO: 57 - protein, 107 aa, synthetic construct
DIQMTQSPSSLSASVGDRVTITCRASQDISNYLNWYQQKPGKAPKLLIYYTSRLHSGVPSRFSGSGSGTDFTFTISSLQYEDIATYYCQQGNTLPPTFGQGTKVEIK

SEQ ID NO: 58 - protein, 26 aa, synthetic construct [sequence omitted]

SEQ ID NO: 59 - protein, 6 aa, synthetic construct
QDISNY

SEQ ID NO: 60 - protein, 17 aa, synthetic construct
LNWYQQKPGKAPKLLIY

SEQ ID NO: 61 - skipped

SEQ ID NO: 62 - protein, 36 aa, synthetic construct
RLHSGVPSRFSGSGSGTDFTFTISSLQYEDIATYYC

SEQ ID NO: 63 - protein, 9 aa, synthetic construct
QQGNTLPPT

SEQ ID NO: 64 - protein, 10 aa, synthetic construct
FGQGTKVEIK

SEQ ID NO: 65 - protein, 117 aa, Mus musculus
QVQLQQPGAELVKPGASVKMSCKTSGYTFTSCNMHWVKQTPGQGLEWIGAVYPGNGDTSYNQKFKGKATLTADKSSSTAYMQLSSLTSEDSAVYYCARGKRDAMDYWGQGTSVTVSS

SEQ ID NO: 66 - protein, 25 aa, Mus musculus
QVQLQQPGAELVKPGASVKMSCKTS

SEQ ID NO: 67 - protein, 8 aa, Mus musculus
GYTFTSCN

SEQ ID NO: 68 - protein, 17 aa, Mus musculus
MHWVKQTPGQGLEWIGA

SEQ ID NO: 69 - protein, 8 aa, Mus musculus
VYPGNGDT

SEQ ID NO: 70 - protein, 38 aa, Mus musculus [sequence omitted]

SEQ ID NO: 71 - protein, 10 aa, Mus musculus
ARGKRDAMDY

SEQ ID NO: 72 - protein, 11 aa, Mus musculus
WGQGTSVTVSS

SEQ ID NO: 73 - protein, 111 aa, Mus musculus
DIVLTQSPASLAVSLGQRATISCRASESVDSYGNSFMHWYQQKPGQPPKLLIYRASNLESGIPARFSGSGSRTDFTLTINPVEADDVATYYCQQSNEDPLTFGAGTKLELK

SEQ ID NO: 74 - protein, 26 aa, Mus musculus
DIVLTQSPASLAVSLGQRATISCRAS

SEQ ID NO: 75 - protein, 10 aa, Mus musculus
ESVDSYGNSF

SEQ ID NO: 76 - protein, 17 aa, Mus musculus
MHWYQQKPGQPPKLLIY

SEQ ID NO: 77 - skipped

SEQ ID NO: 78 - protein, 36 aa, Mus musculus
NLESGIPARFSGSGSRTDFTLTINPVEADDVATYYC

SEQ ID NO: 79 - protein, 9 aa, Mus musculus
QQSNEDPLT

SEQ ID NO: 80 - protein, 10 aa, Mus musculus
FGAGTKLELK

SEQ ID NO: 81 - protein, 117 aa, synthetic construct
QVQLVQSGAEVKKPGASVKVSCKASGYTFTSCNMHWVRQAPGQRLEWIGAVYPGNGDTSYNQKFQGRVTITRDTSASTAYMELSSLRSEDTAVYYCARGKRDAMDYWGQGTLVTVSS

SEQ ID NO: 82 - protein, 25 aa, synthetic construct [sequence omitted]

SEQ ID NO: 83 - protein, 8 aa, synthetic construct
GYTFTSCN

SEQ ID NO: 84 - protein, 17 aa, synthetic construct
MHWVRQAPGQRLEWIGA

SEQ ID NO: 85 - protein, 8 aa, synthetic construct
VYPGNGDT

SEQ ID NO: 86 - protein, 38 aa, synthetic construct
SYNQKFQGRVTITRDTSASTAYMELSSLRSEDTAVYYC

SEQ ID NO: 87 - protein, 10 aa, synthetic construct
ARGKRDAMDY

SEQ ID NO: 88 - protein, 11 aa, synthetic construct
WGQGTLVTVSS

SEQ ID NO: 89 - protein, 117 aa, synthetic construct
QVQLVQSGAEVKKPGASVKVSCKTSGYTFTSCNMHWVRQAPGQRLEWIGAVYPGNGDTSYNQKFQGRVTITRDTSASTAYMELSSLRSEDTAVYYCARGKRDAMDYWGQGTLVTVSS

SEQ ID NO: 90 - protein, 25 aa, synthetic construct
QVQLVQSGAEVKKPGASVKVSCKTS

SEQ ID NO: 91 - protein, 8 aa, synthetic construct
GYTFTSCN

SEQ ID NO: 92 - protein, 17 aa, synthetic construct
MHWVRQAPGQRLEWIGA

SEQ ID NO: 93 - protein, 8 aa, synthetic construct
VYPGNGDT

SEQ ID NO: 94 - protein, 38 aa, synthetic construct; identical to SEQ ID NO: 86

SEQ ID NO: 95 - protein, 10 aa, synthetic construct
ARGKRDAMDY

SEQ ID NO: 96 - protein, 11 aa, synthetic construct
WGQGTLVTVSS

SEQ ID NO: 97 - protein, 111 aa, synthetic construct
DIVMTQTPLSLSVTPGQPASISCRASESVDSYGNSFMHWYLQKPGQPPQLLIYRASNLESGVPDRFSGSGSGTDFTLKISRVEAEDVGVYYCQQSNEDPLTFGQGTKVEIK

SEQ ID NO: 98 - protein, 26 aa, synthetic construct
DIVMTQTPLSLSVTPGQPASISCRAS

SEQ ID NO: 99 - protein, 10 aa, synthetic construct
ESVDSYGNSF

SEQ ID NO: 100 - protein, 17 aa, synthetic construct
MHWYLQKPGQPPQLLIY

SEQ ID NO: 101 - skipped

SEQ ID NO: 102 - protein, 36 aa, synthetic construct
NLESGVPDRFSGSGSGTDFTLKISRVEAEDVGVYYC

SEQ ID NO: 103 - protein, 9 aa, synthetic construct
QQSNEDPLT

SEQ ID NO: 104 - protein, 10 aa, synthetic construct
FGQGTKVEIK

SEQ ID NO: 105 - protein, 111 aa, synthetic construct
DIVMTQTPLSLSVTPGQRASISCRASESVDSYGNSFMHWYLQKPGQPPQLLIYRASNLESGVPDRFSGSGSGTDFTLKISRVEAEDVGVYYCQQSNEDPLTFGQGTKVEIK

SEQ ID NO: 106 - protein, 26 aa, synthetic construct
DIVMTQTPLSLSVTPGQRASISCRAS

SEQ ID NO: 107 - protein, 10 aa, synthetic construct
ESVDSYGNSF

SEQ ID NO: 108 - protein, 17 aa, synthetic construct
MHWYLQKPGQPPQLLIY

SEQ ID NO: 109 - skipped

SEQ ID NO: 110 - protein, 36 aa, synthetic construct; identical to SEQ ID NO: 102

SEQ ID NO: 111 - protein, 9 aa, synthetic construct
QQSNEDPLT

SEQ ID NO: 112 - protein, 10 aa, synthetic construct
FGQGTKVEIK

SEQ ID NO: 113 - protein, 111 aa, synthetic construct
DIVMTQTPLSLSVTPGQRASISCRASESVDSYGNSFMHWYLQKPGQPPQLLIYRASNLESGVPDRFSGSGSGTDFTLTISRVEAEDVGVYYCQQSNEDPLTFGQGTKVEIK

SEQ ID NO: 114 - protein, 26 aa, synthetic construct
DIVMTQTPLSLSVTPGQRASISCRAS

SEQ ID NO: 115 - protein, 10 aa, synthetic construct
ESVDSYGNSF

SEQ ID NO: 116 - protein, 17 aa, synthetic construct
MHWYLQKPGQPPQLLIY

SEQ ID NO: 117 - skipped

SEQ ID NO: 118 - protein, 36 aa, synthetic construct
NLESGVPDRFSGSGSGTDFTLTISRVEAEDVGVYYC

SEQ ID NO: 119 - protein, 9 aa, synthetic construct
QQSNEDPLT

SEQ ID NO: 120 - protein, 10 aa, synthetic construct
FGQGTKVEIK